European Patent Specification EP 3 257 523 B1, published May 20, 2026. Title: USE OF POLYPEPTIDE COMPLEX AS POLYPEPTIDE OR PROTEIN DRUG CARRIER, METHOD, AND FUSION PROTEIN COMPLEX THEREOF. Applicant: Tianjin Institute of Industrial Biotechnology, Chinese Academy of Sciences. The sequence listing filed with the application follows.

SEQUENCE LISTING (32 sequences)

SEQ ID NO: 1 - DNA, 348 bp, Artificial Sequence
  CDS (1)..(348)
atgaaacatcatcatcatcatcatcccatgagcgattacgacatccccactactgagaatctttattttcagggcgccatggctacctcagagctgagctgcgaggtgtcggaggagaactgtgagcgccgggaggccttctgggcagaatggaaggatctgacactgtccacacggcccgaggagggctgctccctgcatgaggaggacacccagagacatgagacctaccaccagcaggggcagtgccaggtgctggtgcagcgctcgccctggctgatgatgcggatgggcatcctcggccgtgggctgcaggagtaccagctgccctaccagcgggtactgccg

SEQ ID NO: 2 - protein, 116 aa, Artificial Sequence
MKHHHHHHPMSDYDIPTTENLYFQGAMATSELSCEVSEENCERREAFWAEWKDLTLSTRPEEGCSLHEEDTQRHETYHQQGQCQVLVQRSPWLMMRMGILGRGLQEYQLPYQRVLP

SEQ ID NO: 3 - DNA, 348 bp, Artificial Sequence
  CDS (1)..(348)
atgaaacatcatcatcatcatcatcccatgagcgattacgacatccccactactgagaatctttattttcagggcgccatggctacctcagagctgagcagcgaggtgtcggaggagaactcggagcgccgggaggccttctgggcagaatggaaggatctgacactgtccacacggcccgaggagggcagctccctgcatgaggaggacacccagagacatgagacctaccaccagcaggggcagagccaggtgctggtgcagcgctcgccctggctgatgatgcggatgggcatcctcggccgtgggctgcaggagtaccagctgccctaccagcgggtactgccg

SEQ ID NO: 4 - protein, 116 aa, Artificial Sequence
MKHHHHHHPMSDYDIPTTENLYFQGAMATSELSSEVSEENSERREAFWAEWKDLTLSTRPEEGSSLHEEDTQRHETYHQQGQSQVLVQRSPWLMMRMGILGRGLQEYQLPYQRVLP

SEQ ID NO: 5 - DNA, 663 bp, Artificial Sequence
  CDS (1)..(663)
atgaaacatcatcatcatcatcatcccatgagcgattacgacatccccactactgagaatctttattttcagggcgccatggccactcaagcaccgacgtttacgcagccgttacaaagcgttgtggtactggagggtagtaccgcaacctttgaggctcacattagtggttttccagttcctgaggtgagctggtttagggatggccaggtgatttccacttccactctgcccggcgtgcagatctcctttagcgatggccgcgctaaactgacgatccccgccgtgactaaagccaacagtggacgatattccctgaaagccaccaatggatctggacaagcgactagtactgctgagcttctcgtgaaagctgagacagcaccacccaacttcgttcaacgactgcagagcatgaccgtgagacaaggaagccaagtgagactccaagtgagagtgactggaatccctacacctgtggtgaagttctaccgggatggagccgaaatccagagctcccttgatttccaaatttcacaagaaggcgacctctacagcttactgattgcagaagcataccctgaggactcagggacctattcagtaaatgccaccaatagcgttggaagagctacttcgactgctgaattactggttcaaggt

SEQ ID NO: 6 - protein, 221 aa, Artificial Sequence
MKHHHHHHPMSDYDIPTTENLYFQGAMATQAPTFTQPLQSVVVLEGSTATFEAHISGFPVPEVSWFRDGQVISTSTLPGVQISFSDGRAKLTIPAVTKANSGRYSLKATNGSGQATSTAELLVKAETAPPNFVQRLQSMTVRQGSQVRLQVRVTGIPTPVVKFYRDGAEIQSSLDFQISQEGDLYSLLIAEAYPEDSGTYSVNATNSVGRATSTAELLVQG

SEQ ID NO: 7 - DNA, 486 bp, Artificial Sequence
  CDS (1)..(486)
atgaaacatcatcatcatcatcatcccatgagcgattacgacatccccactactgagaatctttattttcagcatgcggaaggcacctttaccagcgatgtgagcagctatctggaaggccaggcggcgaaagagtttattgcgtggctggtgaaaggccgtggtggtggtggtggttctggtggtggtggttctggtggtggtggttctgccatggctacctcagagctgagcagcgaggtgtcggaggagaactcggagcgccgggaggccttctgggcagaatggaaggatctgacactgtccacacggcccgaggagggcagctccctgcatgaggaggacacccagagacatgagacctaccaccagcaggggcagagccaggtgctggtgcagcgctcgccctggctgatgatgcggatgggcatcctcggccgtgggctgcaggagtaccagctgccctaccagcgggtactgccgtaa

SEQ ID NO: 8 - protein, 161 aa, Artificial Sequence
MKHHHHHHPMSDYDIPTTENLYFQHAEGTFTSDVSSYLEGQAAKEFIAWLVKGRGGGGGSGGGGSGGGGSAMATSELSSEVSEENSERREAFWAEWKDLTLSTRPEEGSSLHEEDTQRHETYHQQGQSQVLVQRSPWLMMRMGILGRGLQEYQLPYQRVLP

SEQ ID NO: 9 - DNA, 71 bp, Artificial Sequence
ggtggtggtggtggttctggtggtggtggttctggtggtggtggttctgccatggctacctcagagctgag

SEQ ID NO: 10 - DNA, 30 bp, Artificial Sequence
ctgaaaataaagattctcagtagtggggat

SEQ ID NO: 11 - DNA, 53 bp, Artificial Sequence
  misc_feature: 5ˇ-terminal phosphorylation
catgcggaaggcacctttaccagcgatgtgagcagctatctggaaggccaggc

SEQ ID NO: 12 - DNA, 56 bp, Artificial Sequence
  misc_feature: 5ˇ-terminal phosphorylation
gccacggcctttcaccagccacgcaataaactctttcgccgcctggccttccagat

SEQ ID NO: 13 - DNA, 486 bp, Artificial Sequence
  CDS (1)..(486)
atgaaacatcatcatcatcatcatcccatgagcgattacgacatccccactactgagaatctttattttcagcatggcgaaggcacctttaccagcgatgtgagcagctatctggaaggccaggcggcgaaagagtttattgcgtggctggtgaaaggccgtggtggtggtggtggttctggtggtggtggttctggtggtggtggttctgccatggctacctcagagctgagcagcgaggtgtcggaggagaactcggagcgccgggaggccttctgggcagaatggaaggatctgacactgtccacacggcccgaggagggcagctccctgcatgaggaggacacccagagacatgagacctaccaccagcaggggcagagccaggtgctggtgcagcgctcgccctggctgatgatgcggatgggcatcctcggccgtgggctgcaggagtaccagctgccctaccagcgggtactgccgtaa

SEQ ID NO: 14 - protein, 161 aa, Artificial Sequence
MKHHHHHHPMSDYDIPTTENLYFQHGEGTFTSDVSSYLEGQAAKEFIAWLVKGRGGGGGSGGGGSGGGGSAMATSELSSEVSEENSERREAFWAEWKDLTLSTRPEEGSSLHEEDTQRHETYHQQGQSQVLVQRSPWLMMRMGILGRGLQEYQLPYQRVLP

SEQ ID NO: 15 - DNA, 36 bp, Artificial Sequence
aatctttattttcagcatggcgaaggcacctttacc

SEQ ID NO: 16 - DNA, 39 bp, Artificial Sequence
gccatgctgaaaataaagattctcagtagtggggatgtc

SEQ ID NO: 17 - DNA, 783 bp, Artificial Sequence
  CDS (1)..(783)
atgaaacatcatcatcatcatcatccaatgagcgattatgacatccctactagtgaaaatctgtattttcagcatggcgaaggcacgtttacgagtgatgtgtcaagttacctagaaggccaggccgcaaaagagttcattgcttggttagttaaaggtcgtggatccgaagctgctgctaaagaagctgctgctaaagccacccaggctccgacgtttacgcagccattacagagcgttgttgtgctggaaggtagtacagctacctttgaagcacatatctctggctttcctgttccggaagtgtcttggtttcgtgatggtcaggttattagcacctcaaccttaccgggtgtgcaaatttcttttagtgatggtcgcgctaaactgaccattcctgccgtgacaaaagctaattctggtcgctattcactgaaagcaaccaatggtagcggccaggcaacgagtaccgctgaactgctggttaaagccgaaaccgcccctcctaattttgtgcagcgcttacagtctatgaccgttcgtcagggctcacaggttcgcttacaggtgcgcgtgacgggcattcctacaccagttgttaaattttatcgcgatggtgcagaaatccagtctagcttagattttcagatttcacaggaaggcgatctgtatagcctgctgattgccgaagcatatccggaagattctggaacgtatagtgtgaatgcgacaaatagcgtgggtcgcgcaacgagtaccgccgaactgttagttcagggttaa

SEQ ID NO: 18 - protein, 260 aa, Artificial Sequence
MKHHHHHHPMSDYDIPTSENLYFQHGEGTFTSDVSSYLEGQAAKEFIAWLVKGRGSEAAAKEAAAKATQAPTFTQPLQSVVVLEGSTATFEAHISGFPVPEVSWFRDGQVISTSTLPGVQISFSDGRAKLTIPAVTKANSGRYSLKATNGSGQATSTAELLVKAETAPPNFVQRLQSMTVRQGSQVRLQVRVTGIPTPVVKFYRDGAEIQSSLDFQISQEGDLYSLLIAEAYPEDSGTYSVNATNSVGRATSTAELLVQG

SEQ ID NO: 19 - DNA, 1806 bp, Artificial Sequence
  CDS (1)..(1806)
atgaaacatcaccatcaccatcaccccatgagcgattacgacatccccactactgagaatctttattttcagcatggcgaaggcacctttaccagcgatgtgagcagctatctggaaggccaggcggcgaaagagtttattgcgtggctggtgaaaggccgtggtggtggtggtggttctggtggtggtggttctggtggtggtggttctgccatggccactcaagcaccgacgtttacgcagccgttacaaagcgttgtggtactggagggtagtaccgcaacctttgaggctcacattagtggttttccagttcctgaggtgagctggtttagggatggccaggtgatttccacttccactctgcccggcgtgcagatctcctttagcgatggccgcgctaaactgacgatccccgccgtgactaaagccaacagtggacgatattccctgaaagccaccaatggatctggacaagcgactagtactgctgagcttctcgtgaaagctgagacagcaccacccaacttcgttcaacgactgcagagcatgaccgtgagacaaggaagccaagtgagactccaagtgagagtgactggaatccctacacctgtggtgaagttctaccgggatggagccgaaatccagagctcccttgatttccaaatttcacaagaaggcgacctctacagcttactgattgcagaagcataccctgaggactcagggacctattcagtaaatgccaccaatagcgttggaagagctacttcgactgctgaattactggttcaaggttctggttctggttctgctccgggtaccccgggtggtggtggttctggtggtggtggttctggtggtggtggttctatggctacctcagagctgagcagcgaggtgtcggaggagaactcggagcgccgggaggccttctgggcagaatggaaggatctgacactgtccacacggcccgaggagggcagctccctgcatgaggaggacacccagagacatgagacctaccaccagcaggggcagagccaggtgctggtgcagcgctcgccctggctgatgatgcggatgggcatcctcggccgtgggctgcaggagtaccagctgccctaccagcgggtactgccgggtgcttctggtccggctggttctccgaccggttctggtccgggttctgctggttctggtccgggttctgctggtatggccactcaagcaccgacgtttacgcagccgttacaaagcgttgtggtactggagggtagtaccgcaacctttgaggctcacattagtggttttccagttcctgaggtgagctggtttagggatggccaggtgatttccacttccactctgcccggcgtgcagatctcctttagcgatggccgcgctaaactgacgatccccgccgtgactaaagccaacagtggacgatattccctgaaagccaccaatggatctggacaagcgactagtactgctgagcttctcgtgaaagctgagacagcaccacccaacttcgttcaacgactgcagagcatgaccgtgagacaaggaagccaagtgagactccaagtgagagtgactggaatccctacacctgtggtgaagttctaccgggatggagccgaaatccagagctcccttgatttccaaatttcacaagaaggcgacctctacagcttactgattgcagaagcataccctgaggactcagggacctattcagtaaatgccaccaatagcgttggaagagctacttcgactgctgaattactggttcaaggttaa

SEQ ID NO: 20 - protein, 601 aa, Artificial Sequence
MKHHHHHHPMSDYDIPTTENLYFQHGEGTFTSDVSSYLEGQAAKEFIAWLVKGRGGGGGSGGGGSGGGGSAMATQAPTFTQPLQSVVVLEGSTATFEAHISGFPVPEVSWFRDGQVISTSTLPGVQISFSDGRAKLTIPAVTKANSGRYSLKATNGSGQATSTAELLVKAETAPPNFVQRLQSMTVRQGSQVRLQVRVTGIPTPVVKFYRDGAEIQSSLDFQISQEGDLYSLLIAEAYPEDSGTYSVNATNSVGRATSTAELLVQGSGSGSAPGTPGGGGSGGGGSGGGGSMATSELSSEVSEENSERREAFWAEWKDLTLSTRPEEGSSLHEEDTQRHETYHQQGQSQVLVQRSPWLMMRMGILGRGLQEYQLPYQRVLPGASGPAGSPTGSGPGSAGSGPGSAGMATQAPTFTQPLQSVVVLEGSTATFEAHISGFPVPEVSWFRDGQVISTSTLPGVQISFSDGRAKLTIPAVTKANSGRYSLKATNGSGQATSTAELLVKAETAPPNFVQRLQSMTVRQGSQVRLQVRVTGIPTPVVKFYRDGAEIQSSLDFQISQEGDLYSLLIAEAYPEDSGTYSVNATNSVGRATSTAELLVQG

SEQ ID NO: 21 - DNA, 25 bp, Artificial Sequence
cagctctagaaataattttgtttaa

SEQ ID NO: 22 - DNA, 51 bp, Artificial Sequence
cggggtacccggagcagaaccagaaccagaaccttgaaccagtaattcagc

SEQ ID NO: 23 - DNA, 81 bp, Artificial Sequence
tctgctccgggtaccccgggtggtggtggttctggtggtggtggttctggtggtggtggttctatggctacctcagagctg

SEQ ID NO: 24 - DNA, 46 bp, Artificial Sequence
ggtcggagaaccagccggaccagaagcacccggcagtacccgctgg

SEQ ID NO: 25 - DNA, 80 bp, Artificial Sequence
ccggctggttctccgaccggttctggtccgggttctgctggttctggtccgggttctgctggtatggccactcaagcacc

SEQ ID NO: 26 - DNA, 20 bp, Artificial Sequence
attcggatccggtaccttaa

SEQ ID NO: 27 - DNA, 399 bp, Artificial Sequence
  CDS (1)..(399)
atgaaacatcatcatcatcatcatcccatgagcgattacgacatccccactactgagaatctttattttcagggcgccatggctacctcagagctgagcagcgaggtgtcggaggagaactcggaggcaggttgcaagaactttttttggaaaacctttacctcttgcggtggtcgccgggaggccttctgggcagaatggaaggatctgacactgtccacacggcccgaggagggcagctccctgcatgaggaggacacccagagacatgagacctaccaccagcaggggcagagccaggtgctggtgcagcgctcgccctggctgatgatgcggatgggcatcctcggccgtgggctgcaggagtaccagctgccctaccagcgggtactgccgtaa

SEQ ID NO: 28 - protein, 132 aa, Artificial Sequence
MKHHHHHHPMSDYDIPTTENLYFQGAMATSELSSEVSEENSEAGCKNFFWKTFTSCGGRREAFWAEWKDLTLSTRPEEGSSLHEEDTQRHETYHQQGQSQVLVQRSPWLMMRMGILGRGLQEYQLPYQRVLP

SEQ ID NO: 29 - DNA, 714 bp, Artificial Sequence
  CDS (1)..(714)
atgaaacatcaccatcaccatcaccccatgagcgattacgacatccccactactgagaatctttattttcagggcgccatggccactcaagcaccgacgtttacgcagccgttacaaagcgttgtggtactggagggtagtaccgcaacctttgaggctcacattagtggttttccagttcctgaggtgagctggtttagggatggccaggtgatttccacttccactctgcccggcgtgcagatctcctttagcgatggccgcgctaaactgacgatccccgccgtgactaaagccaacagtggacgatattccctgaaagccaccaatggatctggacaagcgactagtactgctgagcttctcgtgaaagctgagacagcaccacccaacttcgttcaacgactgcagagcatgaccgtgagacaaggaagccaagtgagactccaagtgagagtgactggaatccctacacctgtggtgaagttctaccgggatggagccgaaatcgcaggttgcaagaactttttttggaaaacctttacctcttgcggtgcccagagctcccttgatttccaaatttcacaagaaggcgacctctacagcttactgattgcagaagcataccctgaggactcagggacctattcagtaaatgccaccaatagcgttggaagagctacttcgactgctgaattactggttcaaggttaa

SEQ ID NO: 30 - protein, 237 aa, Artificial Sequence
MKHHHHHHPMSDYDIPTTENLYFQGAMATQAPTFTQPLQSVVVLEGSTATFEAHISGFPVPEVSWFRDGQVISTSTLPGVQISFSDGRAKLTIPAVTKANSGRYSLKATNGSGQATSTAELLVKAETAPPNFVQRLQSMTVRQGSQVRLQVRVTGIPTPVVKFYRDGAEIAGCKNFFWKTFTSCGAQSSLDFQISQEGDLYSLLIAEAYPEDSGTYSVNATNSVGRATSTAELLVQG

SEQ ID NO: 31 - DNA, 462 bp, Artificial Sequence
  CDS (1)..(462)
atgaaacatcaccatcaccatcaccccatgagcgattacgacatccccactactgagaatctttattttcagggcgccatggctacctcagagctgagcagcgaggtgtcggaggagaactcggagcgccgggaggccttctgggcagaatggaaggatctgacactgtccacacggcccgaggagggcagctccctgcatgaggaggacacccagagacatgagacctaccaccagcaggggcagagccaggtgctggtgcagcgctcgccctggctgatgatgcggatgggcatcctcggccgtgggctgcaggagtaccagctgccctaccagcgggtactgccgggtagcggtattaaaccggaagcaccgggtgaagatgcaagcccggaagaactgaatcgttattatgcaagcctgcgccattatctgaatctggttacccgccagcgctattaa

SEQ ID NO: 32 - protein, 153 aa, Artificial Sequence
MKHHHHHHPMSDYDIPTTENLYFQGAMATSELSSEVSEENSERREAFWAEWKDLTLSTRPEEGSSLHEEDTQRHETYHQQGQSQVLVQRSPWLMMRMGILGRGLQEYQLPYQRVLPGSGIKPEAPGEDASPEELNRYYASLRHYLNLVTRQRY